European Patent Application EP 4 620 970 A1, published September 24, 2025. Title: Porin Monomer, Porin, and Mutant and Application Thereof. Applicant: BGI SHENZHEN. The sequence listing filed with the application follows.

SEQUENCE LISTING (19 sequences)

SEQ ID NO: 1 - protein, 319 aa, synthetic construct
  source 1..319: note = The monomer of wild-type porin BCP58
MKSYMSQISRKRQLMVCLLSLTFAGCVSTPIPPSLESARLTSRTSTYDDLRALPVPKGKIVVSLYKFNDQTGQYKPSPASSFSTAVTQGATAMLVQALHESGWFIVLEREGLQNLLTERKIIRAAQKKPNTPVNNADDLPSLLAANVLIEGGVIAYESNVKTGGAGARFLGIGFSEQYRVDQVTVNLRAINVSTGRILHNVSTTKTILSKELQSSVYKFVEYKELLELEAGTTTNEPTQMCVRAAIEAAVIHMLVDGLENRSWSLASESDVSNPVIKRYSEETPKVVIKSAALTSPSDNSLAVMPSATNYYDEIMSGVK

SEQ ID NO: 2 - protein, 319 aa, synthetic construct
  source 1..319: note = The monomer of porin BCP58 mutant 1
MKSYMSQISRKRQLMVCLLSLTFAGCVSTPIPPSLESARLTSRTSTYDDLRALPVPKGKIVVSLYKFNDQTGQYKPAPASSQSTAVTQGATAMLVQALHESGWFIVLEREGLQNLLTERKIIRAAQKKPNTPVNNADDLPSLLAANVLIEGGVIAYESNVKTGGAGARFLGIGFSEQYRVDQVTVNLRAINVSTGRILHNVSTTKTILSKELQSSVYKFVEYKELLELEAGTTTNEPTQMCVRAAIEAAVIHMLVDGLENRSWSLASESDVSNPVIKRYSEETPKVVIKSAALTSPSDNSLAVMPSATNYYDEIMSGVK

SEQ ID NO: 3 - protein, 319 aa, synthetic construct
  source 1..319: note = The monomer of porin BCP58 mutant 2
MKSYMSQISRKRQLMVCLLSLTFAGCVSTPIPPSLESARLTSRTSTYDDLRALPVPKGKIVVSLYKFNDQTGQYKPSPASNASTAVTQGATAMLVQALHESGWFIVLEREGLQNLLTERKIIRAAQKKPNTPVNNADDLPSLLAANVLIEGGVIAYESNVKTGGAGARFLGIGFSEQYRVDQVTVNLRAINVSTGRILHNVSTTKTILSKELQSSVYKFVEYKELLELEAGTTTNEPTQMCVRAAIEAAVIHMLVDGLENRSWSLASESDVSNPVIKRYSEETPKVVIKSAALTSPSDNSLAVMPSATNYYDEIMSGVK

SEQ ID NO: 4 - protein, 319 aa, synthetic construct
  source 1..319: note = The monomer of porin BCP58 mutant 3
MKSYMSQISRKRQLMVCLLSLTFAGCVSTPIPPSLESARLTSRTSTYDDLRALPVPKGKIVVSLYKFNDQTGQYKPSPASNASTAVTQGATAMLVQALHESGWFIVLEREGLQNLLTERNIIRAAQKKPNTPVNNADDLPSLLAANVLIEGGVIAYESNVKTGGAGARFLGIGFSEQYRVDQVTVNLRAINVSTGRILHNVSTTKTILSKELQSSVYKFVEYKELLELEAGTTTNEPTQMCVRAAIEAAVIHMLVDGLENRSWSLASESDVSNPVIKRYSEETPKVVIKSAALTSPSDNSLAVMPSATNYYDEIMSGVK

SEQ ID NO: 5 - protein, 319 aa, synthetic construct
  source 1..319: note = The monomer of porin BCP58 mutant 4
MKSYMSQISRKRQLMVCLLSLTFAGCVSTPIPPSLESARLTSRTSTYDDLRALPVPKGKIVVSLYKFNDQTGQYKPSPASNASTAVTQGATAMLVQALHESGWFIVLEREGLQNLLTERKIIRAAQSKPNTPVNNADDLPSLLAANVLIEGGVIAYESNVKTGGAGARFLGIGFSEQYRVDQVTVNLRAINVSTGRILHNVSTTKTILSKELQSSVYKFVEYKELLELEAGTTTNEPTQMCVRAAIEAAVIHMLVDGLENRSWSLASESDVSNPVIKRYSEETPKVVIKSAALTSPSDNSLAVMPSATNYYDEIMSGVK

SEQ ID NO: 6 - protein, 319 aa, synthetic construct
  source 1..319: note = The monomer of porin BCP58 mutant 5
MKSYMSQISRKRQLMVCLLSLTFAGCVSTPIPPSLESARLTSRTSTYDDLRALPVPKGKIVVSLYKFNDQTGQYKPSPASSFSTAVTQGATAMLVQALHESGWFIVLEREGLQNLLTERKIIRAAQKKPNTPVNNADDLPSLLAANVLIEGGVIAYESNVKTGGAGARFLGIGFSIQYRVDQVTVNLRAINVSTGRILHNVSTTKTILSKELQSSVYKFVEYKELLELEAGTTTNEPTQMCVRAAIEAAVIHMLVDGLENRSWSLASESDVSNPVIKRYSEETPKVVIKSAALTSPSDNSLAVMPSATNYYDEIMSGVK

SEQ ID NO: 7 - DNA, 960 bp, synthetic construct
  source 1..960: mol_type = other DNA; note = The nucleotide sequence encoding the monomer of wild-type porin BCP58
atgaaaagctatatgagccagattagccgtaaacgccagctgatggtttgtctgctgagcctgacctttgcaggttgtgttagcaccccgattccgccgagtctggaaagtgcacgtttaacaagtcgtaccagcacctatgatgatctgcgtgcactgccggttccgaaaggtaaaattgttgttagcctgtataagttcaacgaccagaccggtcagtataagccgagcccggcaagtagctttagcaccgcagttacccagggtgcaaccgcaatgctggttcaggcactgcatgaaagcggttggtttattgttctggaacgtgaaggtctgcagaatctgctgaccgaacgtaaaattattcgcgcagcacagaaaaaaccgaataccccggttaataatgccgatgatctgccgagcctgctggcagcaaatgttctgattgaaggtggtgttattgcctatgaaagcaatgttaaaaccggcggcgcaggtgcacgttttctgggtattggttttagcgaacagtatcgggttgatcaggttaccgttaatctgcgtgcaattaatgttagcaccggtcgtattctgcataatgttagcaccaccaaaaccattctgagcaaagaactgcagagcagcgtttataaatttgttgagtataaggagctgctggagctggaggcaggtaccaccacaaatgaaccgacccagatgtgtgttcgtgcagcaattgaagcagcagttattcacatgctggttgacggtctggaaaatcgtagctggagcctggcaagcgaaagcgatgttagcaatccggttattaaacgttatagcgaggaaaccccgaaagttgttattaaaagcgcagcactgaccagcccgagcgataatagcctggcagttatgccgagcgcaaccaattattatgatgaaattatgagcggcgtgaagtaa

SEQ ID NO: 8 - DNA, 960 bp, synthetic construct
  source 1..960: mol_type = other DNA; note = The nucleotide sequence encoding the monomer of porin BCP58 mutant 1
atgaaaagctatatgagccagattagccgtaaacgccagctgatggtttgtctgctgagcctgacctttgcaggttgtgttagcaccccgattccgccgagtctggaaagtgcacgtttaacaagtcgtaccagcacctatgatgatctgcgtgcactgccggttccgaaaggtaaaattgttgttagcctgtataagttcaacgaccagaccggtcagtataagccggcaccggcaagtagccagagcaccgcagttacccagggtgcaaccgcaatgctggttcaggcactgcatgaaagcggttggtttattgttctggaacgtgaaggtctgcagaatctgctgaccgaacgtaaaattattcgcgcagcacagaaaaaaccgaataccccggttaataatgccgatgatctgccgagcctgctggcagcaaatgttctgattgaaggtggtgttattgcctatgaaagcaatgttaaaaccggcggcgcaggtgcacgttttctgggtattggttttagcgaacagtatcgggttgatcaggttaccgttaatctgcgtgcaattaatgttagcaccggtcgtattctgcataatgttagcaccaccaaaaccattctgagcaaagaactgcagagcagcgtttataaatttgttgagtataaggagctgctggagctggaggcaggtaccaccacaaatgaaccgacccagatgtgtgttcgtgcagcaattgaagcagcagttattcacatgctggttgacggtctggaaaatcgtagctggagcctggcaagcgaaagcgatgttagcaatccggttattaaacgttatagcgaggaaaccccgaaagttgttattaaaagcgcagcactgaccagcccgagcgataatagcctggcagttatgccgagcgcaaccaattattatgatgaaattatgagcggcgtgaagtaa

SEQ ID NO: 9 - DNA, 960 bp, synthetic construct
  source 1..960: mol_type = other DNA; note = The nucleotide sequence encoding the monomer of porin BCP58 mutant 2
atgaaaagctatatgagccagattagccgtaaacgccagctgatggtttgtctgctgagcctgacctttgcaggttgtgttagcaccccgattccgccgagtctggaaagtgcacgtttaacaagtcgtaccagcacctatgatgatctgcgtgcactgccggttccgaaaggtaaaattgttgttagcctgtataagttcaacgaccagaccggtcagtataagccgagcccggcaagtaatgcaagcaccgcagttacccagggtgcaaccgcaatgctggttcaggcactgcatgaaagcggttggtttattgttctggaacgtgaaggtctgcagaatctgctgaccgaacgtaaaattattcgcgcagcacagaaaaaaccgaataccccggttaataatgccgatgatctgccgagcctgctggcagcaaatgttctgattgaaggtggtgttattgcctatgaaagcaatgttaaaaccggcggcgcaggtgcacgttttctgggtattggttttagcgaacagtatcgggttgatcaggttaccgttaatctgcgtgcaattaatgttagcaccggtcgtattctgcataatgttagcaccaccaaaaccattctgagcaaagaactgcagagcagcgtttataaatttgttgagtataaggagctgctggagctggaggcaggtaccaccacaaatgaaccgacccagatgtgtgttcgtgcagcaattgaagcagcagttattcacatgctggttgacggtctggaaaatcgtagctggagcctggcaagcgaaagcgatgttagcaatccggttattaaacgttatagcgaggaaaccccgaaagttgttattaaaagcgcagcactgaccagcccgagcgataatagcctggcagttatgccgagcgcaaccaattattatgatgaaattatgagcggcgtgaagtaa

SEQ ID NO: 10 - DNA, 960 bp, synthetic construct
  source 1..960: mol_type = other DNA; note = The nucleotide sequence encoding the monomer of porin BCP58 mutant 3
atgaaaagctatatgagccagattagccgtaaacgccagctgatggtttgtctgctgagcctgacctttgcaggttgtgttagcaccccgattccgccgagtctggaaagtgcacgtttaacaagtcgtaccagcacctatgatgatctgcgtgcactgccggttccgaaaggtaaaattgttgttagcctgtataagttcaacgaccagaccggtcagtataagccgagcccggcaagtaatgcaagcaccgcagttacccagggtgcaaccgcaatgctggttcaggcactgcatgaaagcggttggtttattgttctggaacgtgaaggtctgcagaatctgctgaccgaacgtaatattattcgcgcagcacagaaaaaaccgaataccccggttaataatgccgatgatctgccgagcctgctggcagcaaatgttctgattgaaggtggtgttattgcctatgaaagcaatgttaaaaccggcggcgcaggtgcacgttttctgggtattggttttagcgaacagtatcgggttgatcaggttaccgttaatctgcgtgcaattaatgttagcaccggtcgtattctgcataatgttagcaccaccaaaaccattctgagcaaagaactgcagagcagcgtttataaatttgttgagtataaggagctgctggagctggaggcaggtaccaccacaaatgaaccgacccagatgtgtgttcgtgcagcaattgaagcagcagttattcacatgctggttgacggtctggaaaatcgtagctggagcctggcaagcgaaagcgatgttagcaatccggttattaaacgttatagcgaggaaaccccgaaagttgttattaaaagcgcagcactgaccagcccgagcgataatagcctggcagttatgccgagcgcaaccaattattatgatgaaattatgagcggcgtgaagtaa

SEQ ID NO: 11 - DNA, 960 bp, synthetic construct
  source 1..960: mol_type = other DNA; note = The nucleotide sequence encoding the monomer of porin BCP58 mutant 4
atgaaaagctatatgagccagattagccgtaaacgccagctgatggtttgtctgctgagcctgacctttgcaggttgtgttagcaccccgattccgccgagtctggaaagtgcacgtttaacaagtcgtaccagcacctatgatgatctgcgtgcactgccggttccgaaaggtaaaattgttgttagcctgtataagttcaacgaccagaccggtcagtataagccgagcccggcaagtaatgcaagcaccgcagttacccagggtgcaaccgcaatgctggttcaggcactgcatgaaagcggttggtttattgttctggaacgtgaaggtctgcagaatctgctgaccgaacgtaaaattattcgcgcagcacagagcaaaccgaataccccggttaataatgccgatgatctgccgagcctgctggcagcaaatgttctgattgaaggtggtgttattgcctatgaaagcaatgttaaaaccggcggcgcaggtgcacgttttctgggtattggttttagcgaacagtatcgggttgatcaggttaccgttaatctgcgtgcaattaatgttagcaccggtcgtattctgcataatgttagcaccaccaaaaccattctgagcaaagaactgcagagcagcgtttataaatttgttgagtataaggagctgctggagctggaggcaggtaccaccacaaatgaaccgacccagatgtgtgttcgtgcagcaattgaagcagcagttattcacatgctggttgacggtctggaaaatcgtagctggagcctggcaagcgaaagcgatgttagcaatccggttattaaacgttatagcgaggaaaccccgaaagttgttattaaaagcgcagcactgaccagcccgagcgataatagcctggcagttatgccgagcgcaaccaattattatgatgaaattatgagcggcgtgaagtaa

SEQ ID NO: 12 - DNA, 960 bp, synthetic construct
  source 1..960: mol_type = other DNA; note = The nucleotide sequence encoding the monomer of porin BCP58 mutant 5
atgaaaagctatatgagccagattagccgtaaacgccagctgatggtttgtctgctgagcctgacctttgcaggttgtgttagcaccccgattccgccgagtctggaaagtgcacgtttaacaagtcgtaccagcacctatgatgatctgcgtgcactgccggttccgaaaggtaaaattgttgttagcctgtataagttcaacgaccagaccggtcagtataagccgagcccggcaagtagctttagcaccgcagttacccagggtgcaaccgcaatgctggttcaggcactgcatgaaagcggttggtttattgttctggaacgtgaaggtctgcagaatctgctgaccgaacgtaaaattattcgcgcagcacagaaaaaaccgaataccccggttaataatgccgatgatctgccgagcctgctggcagcaaatgttctgattgaaggtggtgttattgcctatgaaagcaatgttaaaaccggcggcgcaggtgcacgttttctgggtattggttttagcattcagtatcgggttgatcaggttaccgttaatctgcgtgcaattaatgttagcaccggtcgtattctgcataatgttagcaccaccaaaaccattctgagcaaagaactgcagagcagcgtttataaatttgttgagtataaggagctgctggagctggaggcaggtaccaccacaaatgaaccgacccagatgtgtgttcgtgcagcaattgaagcagcagttattcacatgctggttgacggtctggaaaatcgtagctggagcctggcaagcgaaagcgatgttagcaatccggttattaaacgttatagcgaggaaaccccgaaagttgttattaaaagcgcagcactgaccagcccgagcgataatagcctggcagttatgccgagcgcaaccaattattatgatgaaattatgagcggcgtgaagtaa

SEQ ID NO: 13 - DNA, 40 bp, synthetic construct
  source 1..40: mol_type = other DNA; note = S1
tttttttttttttttttttttttttttttttttttttttt

SEQ ID NO: 14 - DNA, 28 bp, synthetic construct
  source 1..28: mol_type = other DNA; note = S2
ggttgtttctgttggtgctgatattgct

SEQ ID NO: 15 - DNA, 45 bp, synthetic construct
  source 1..45: mol_type = other DNA; note = The antisense strand of the adapter sequence
gcaatatcagcaccaacagaaacaacctttgaggcgagcggtcaa

SEQ ID NO: 16 - DNA, 2710 bp, synthetic construct
  source 1..2710: mol_type = other DNA; note = pUC57
tcgcgcgtttcggtgatgacggtgaaaacctctgacacatgcagctcccggagacggtcacagcttgtctgtaagcggatgccgggagcagacaagcccgtcagggcgcgtcagcgggtgttggcgggtgtcggggctggcttaactatgcggcatcagagcagattgtactgagagtgcaccatatgcggtgtgaaataccgcacagatgcgtaaggagaaaataccgcatcaggcgccattcgccattcaggctgcgcaactgttgggaagggcgatcggtgcgggcctcttcgctattacgccagctggcgaaagggggatgtgctgcaaggcgattaagttgggtaacgccagggttttcccagtcacgacgttgtaaaacgacggccagtgaattcgagctcggtacctcgcgaatgcatctagatatcggatcccgggcccgtcgactgcagaggcctgcatgcaagcttggcgtaatcatggtcatagctgtttcctgtgtgaaattgttatccgctcacaattccacacaacatacgagccggaagcataaagtgtaaagcctggggtgcctaatgagtgagctaactcacattaattgcgttgcgctcactgcccgctttccagtcgggaaacctgtcgtgccagctgcattaatgaatcggccaacgcgcggggagaggcggtttgcgtattgggcgctcttccgcttcctcgctcactgactcgctgcgctcggtcgttcggctgcggcgagcggtatcagctcactcaaaggcggtaatacggttatccacagaatcaggggataacgcaggaaagaacatgtgagcaaaaggccagcaaaaggccaggaaccgtaaaaaggccgcgttgctggcgtttttccataggctccgcccccctgacgagcatcacaaaaatcgacgctcaagtcagaggtggcgaaacccgacaggactataaagataccaggcgtttccccctggaagctccctcgtgcgctctcctgttccgaccctgccgcttaccggatacctgtccgcctttctcccttcgggaagcgtggcgctttctcatagctcacgctgtaggtatctcagttcggtgtaggtcgttcgctccaagctgggctgtgtgcacgaaccccccgttcagcccgaccgctgcgccttatccggtaactatcgtcttgagtccaacccggtaagacacgacttatcgccactggcagcagccactggtaacaggattagcagagcgaggtatgtaggcggtgctacagagttcttgaagtggtggcctaactacggctacactagaagaacagtatttggtatctgcgctctgctgaagccagttaccttcggaaaaagagttggtagctcttgatccggcaaacaaaccaccgctggtagcggtggtttttttgtttgcaagcagcagattacgcgcagaaaaaaaggatctcaagaagatcctttgatcttttctacggggtctgacgctcagtggaacgaaaactcacgttaagggattttggtcatgagattatcaaaaaggatcttcacctagatccttttaaattaaaaatgaagttttaaatcaatctaaagtatatatgagtaaacttggtctgacagttaccaatgcttaatcagtgaggcacctatctcagcgatctgtctatttcgttcatccatagttgcctgactccccgtcgtgtagataactacgatacgggagggcttaccatctggccccagtgctgcaatgataccgcgagacccacgctcaccggctccagatttatcagcaataaaccagccagccggaagggccgagcgcagaagtggtcctgcaactttatccgcctccatccagtctattaattgttgccgggaagctagagtaagtagttcgccagttaatagtttgcgcaacgttgttgccattgctacaggcatcgtggtgtcacgctcgtcgtttggtatggcttcattcagctccggttcccaacgatcaaggcgagttacatgatcccccatgttgtgcaaaaaagcggttagctccttcggtcctccgatcgttgtcagaagtaagttggccgcagtgttatcactcatggttatggcagcactgcataattctcttactgtcatgccatccgtaagatgcttttctgtgactggtgagtactcaaccaagtcattctgagaatagtgtatgcggcgaccgagttgctcttgcccggcgtcaatacgggataataccgcgccacatagcagaactttaaaagtgctcatcattggaaaacgttcttcggggcgaaaactctcaaggatcttaccgctgttgagatccagttcgatgtaacccactcgtgcacccaactgatcttcagcatcttttactttcaccagcgtttctgggtgagcaaaaacaggaaggcaaaatgccgcaaaaaagggaataagggcgacacggaaatgttgaatactcatactcttcctttttcaatattattgaagcatttatcagggttattgtctcatgagcggatacatatttgaatgtatttagaaaaataaacaaataggggttccgcgcacatttccccgaaaagtgccacctgacgtctaagaaaccattattatcatgacattaacctataaaaataggcgtatcacgaggccctttcgtc

SEQ ID NO: 17 - protein, 454 aa, synthetic construct
  source 1..454: note = BCH105
MKHDLSSATEEQRYIFTDFIKQAQLALKGDSDYEVFAIQGFAGSGKTWLSALIIDELLELGMKVAVTSPTHKAVRVSLNMLKNNGIDTNSPLMYPGTIHHFLNLKLDHGFADDGTACNVTTKAKLVVNKFNEALEYVDVLIVDEASMVSGELYDHALKTLGDRAKIILFIGDSYQLLPVDDEDSSIFLKDDIFHYKLTKVVRQAEDNIIIAKSQELIKAMDQKTYYPSVNDYFVNITEDTEGIKLLKSNVELFELYFSDFKDKMTGAYTNKVVNQFNEYIRYTLYQETKFIADKDELVFQETYTDSKGNIIVSNGEIIEVATAKLTTDIDKFKIWKIVSKKNELGEAVRFNVLDPSSYNEFNDLLDKYCADAKIAKGYDRSKAWKKYFKLKEKYAKVRYNFSSTIHKLQGSTYQNMYFDMRGLDYFYRMNRDNVLRLVYVGITRASDQVFILQD

SEQ ID NO: 18 - DNA, 15 bp, synthetic construct
  source 1..15: mol_type = other DNA; note = The sequence of the single-stranded DNA with cholesterol at the 5' end
ttgaccgctcgcctc

SEQ ID NO: 19 - DNA, 24 bp, synthetic construct
  source 1..24: mol_type = other DNA; note = QC DNA
ttttttttttggtggtgtggttgg